European Patent Application EP 4 530 300 A1, published April 2, 2025. Title: TREFOIL FACTOR 2/INTERFERON α2 FUSION PROTEIN AND APPLICATION THEREOF IN PREVENTION AND TREATMENT OF VIRAL INFECTIOUS DISEASES. Applicant: Fudan University. Application EP 22943010.3. The sequence listing filed with the application follows.

SEQUENCE LISTING (14 sequences)

SEQ ID NO: 1 - DNA, 1554 bp, Artificial
  TFF2-G4S-IFNα2-Fc mRNA coding sequence
gagaagcctagcccttgccagtgcagcagactgtctcctcacaaccgcacaaactgcggcttccctggcattacatccgaccagtgcttcgacaacggctgctgcttcgactctagcgtgacaggcgtgccttggtgcttccacccactgccaaagcaggagtccgaccagtgcgtgatggaggtgagcgaccgccggaactgcggctaccccggcattagccccgaggagtgcgcctcccggaagtgctgcttcagcaacttcattttcgaggtgccttggtgcttcttccctaagtccgtggaggactgccactacggcggcggcggctctggcggcggcggctctggcggcggcggctcttgcgacctcccacagacccactctctgggctctcgcagaacactgatgctcctcgcccagatgagacggattagcctgttctcttgcctcaaggacaggcacgacttcggcttccctcaggaggagttcggcaaccagttccagaaggccgagaccattccagtgctgcacgagatgattcagcagattttcaacctgttcagcaccaaggactctagcgccgcctgggacgagaccctcctcgacaagttctacacagagctgtaccagcagctgaacgacctcgaggcctgcgtgattcagggcgtgggcgtgacagagaccccactcatgaaggaggactccattctggccgtgagaaagtacttccagcgcattacactgtacctgaaggagaagaagtactctccatgcgcctgggaggtggtgcgcgccgagattatgagatctttcagcctgagcacaaacctgcaggagtccctcagatctaaggaggagccaaagtcttgcgacaagacccacacatgcccaccttgccccgcccccgagctcctgggcggcccatctgtgttcctgttcccacctaagccaaaggacacactcatgatttcccgtacacctgaggtgacatgcgtggtggtggacgtgtctcacgaggaccccgaggtgaagttcaactggtacgtggacggcgtggaggtgcacaacgccaagaccaagcctagagaggagcagtacaactctacataccgggtggtgtctgtgctcaccgtgctgcaccaggactggctgaacggcaaggagtacaagtgcaaggtgtctaacaaggccctccccgcccctattgagaagacaatttctaaggccaagggccagcctagagagccacaggtgtacacactgccaccatctcgggacgagctgacaaagaaccaggtgtctctgacatgcctcgtgaagggcttctacccatctgacatcgccgtggagtgggagtctaacggccagcccgagaacaactacaagacaacacctccagtgctcgactccgacggctctttcttcctgtactctaagctcaccgtggacaagagccgctggcagcagggcaacgtgttctcttgcagcgtgatgcacgaggccctgcacaaccactacacacagaagtccctgtctctgtccccaggcaag

SEQ ID NO: 2 - protein, 518 aa, Artificial
  TFF2-G4S-IFNα2-Fc amino acid sequence
EKPSPCQCSRLSPHNRTNCGFPGITSDQCFDNGCCFDSSVTGVPWCFHPLPKQESDQCVMEVSDRRNCGYPGISPEECASRKCCFSNFIFEVPWCFFPKSVEDCHYGGGGSGGGGSGGGGSCDLPQTHSLGSRRTLMLLAQMRRISLFSCLKDRHDFGFPQEEFGNQFQKAETIPVLHEMIQQIFNLFSTKDSSAAWDETLLDKFYTELYQQLNDLEACVIQGVGVTETPLMKEDSILAVRKYFQRITLYLKEKKYSPCAWEVVRAEIMRSFSLSTNLQESLRSKEEPKSCDKTHTCPPCPAPELLGGPSVFLFPPKPKDTLMISRTPEVTCVVVDVSHEDPEVKFNWYVDGVEVHNAKTKPREEQYNSTYRVVSVLTVLHQDWLNGKEYKCKVSNKALPAPIEKTISKAKGQPREPQVYTLPPSRDELTKNQVSLTCLVKGFYPSDIAVEWESNGQPENNYKTTPPVLDSDGSFFLYSKLTVDKSRWQQGNVFSCSVMHEALHNHYTQKSLSLSPGK

SEQ ID NO: 3 - DNA, 1917 bp, Artificial
  2xTFF2-G4S-IFNα2-Fc mRNA coding sequence
gagaagcctagcccttgccagtgcagcagactgtctcctcacaaccgcacaaactgcggcttccctggcattacatccgaccagtgcttcgacaacggctgctgcttcgactctagcgtgacaggcgtgccttggtgcttccacccactgccaaagcaggagtccgaccagtgcgtgatggaggtgagcgaccgccggaactgcggctaccccggcattagccccgaggagtgcgcctcccggaagtgctgcttcagcaacttcattttcgaggtgccttggtgcttcttccctaagtccgtggaggactgccactacggcggcggcggctctggcggcggcggctctggcggcggcggctctgagaagcctagcccttgccagtgcagcagactgtctcctcacaaccgcacaaactgcggcttccctggcattacatccgaccagtgcttcgacaacggctgctgcttcgactctagcgtgacaggcgtgccttggtgcttccacccactgccaaagcaggagtccgaccagtgcgtgatggaggtgagcgaccgccggaactgcggctaccccggcattagccccgaggagtgcgcctcccggaagtgctgcttcagcaacttcattttcgaggtgccttggtgcttcttccctaagtccgtggaggactgccactacggcggcggcggctctggcggcggcggctctggcggcggcggctcttgcgacctcccacagacccactctctgggctctcgcagaacactgatgctcctcgcccagatgagacggattagcctgttctcttgcctcaaggacaggcacgacttcggcttccctcaggaggagttcggcaaccagttccagaaggccgagaccattccagtgctgcacgagatgattcagcagattttcaacctgttcagcaccaaggactctagcgccgcctgggacgagaccctcctcgacaagttctacacagagctgtaccagcagctgaacgacctcgaggcctgcgtgattcagggcgtgggcgtgacagagaccccactcatgaaggaggactccattctggccgtgagaaagtacttccagcgcattacactgtacctgaaggagaagaagtactctccatgcgcctgggaggtggtgcgcgccgagattatgagatctttcagcctgagcacaaacctgcaggagtccctcagatctaaggaggagccaaagtcttgcgacaagacccacacatgcccaccttgccccgcccccgagctcctgggcggcccatctgtgttcctgttcccacctaagccaaaggacacactcatgatttcccgtacacctgaggtgacatgcgtggtggtggacgtgtctcacgaggaccccgaggtgaagttcaactggtacgtggacggcgtggaggtgcacaacgccaagaccaagcctagagaggagcagtacaactctacataccgggtggtgtctgtgctcaccgtgctgcaccaggactggctgaacggcaaggagtacaagtgcaaggtgtctaacaaggccctccccgcccctattgagaagacaatttctaaggccaagggccagcctagagagccacaggtgtacacactgccaccatctcgggacgagctgacaaagaaccaggtgtctctgacatgcctcgtgaagggcttctacccatctgacatcgccgtggagtgggagtctaacggccagcccgagaacaactacaagacaacacctccagtgctcgactccgacggctctttcttcctgtactctaagctcaccgtggacaagagccgctggcagcagggcaacgtgttctcttgcagcgtgatgcacgaggccctgcacaaccactacacacagaagtccctgtctctgtccccaggcaag

SEQ ID NO: 4 - protein, 639 aa, Artificial
  2xTFF2-G4S-IFNα2-Fc amino acid sequence
EKPSPCQCSRLSPHNRTNCGFPGITSDQCFDNGCCFDSSVTGVPWCFHPLPKQESDQCVMEVSDRRNCGYPGISPEECASRKCCFSNFIFEVPWCFFPKSVEDCHYGGGGSGGGGSGGGGSEKPSPCQCSRLSPHNRTNCGFPGITSDQCFDNGCCFDSSVTGVPWCFHPLPKQESDQCVMEVSDRRNCGYPGISPEECASRKCCFSNFIFEVPWCFFPKSVEDCHYGGGGSGGGGSGGGGSCDLPQTHSLGSRRTLMLLAQMRRISLFSCLKDRHDFGFPQEEFGNQFQKAETIPVLHEMIQQIFNLFSTKDSSAAWDETLLDKFYTELYQQLNDLEACVIQGVGVTETPLMKEDSILAVRKYFQRITLYLKEKKYSPCAWEVVRAEIMRSFSLSTNLQESLRSKEEPKSCDKTHTCPPCPAPELLGGPSVFLFPPKPKDTLMISRTPEVTCVVVDVSHEDPEVKFNWYVDGVEVHNAKTKPREEQYNSTYRVVSVLTVLHQDWLNGKEYKCKVSNKALPAPIEKTISKAKGQPREPQVYTLPPSRDELTKNQVSLTCLVKGFYPSDIAVEWESNGQPENNYKTTPPVLDSDGSFFLYSKLTVDKSRWQQGNVFSCSVMHEALHNHYTQKSLSLSPGK

SEQ ID NO: 5 - DNA, 1554 bp, Artificial
  IFNα2-G4S-TFF2-Fc mRNA coding sequence
tgcgacctgcctcagacccactctctgggctctcgcagaacactcatgctcctcgcccagatgagacggatttctctgttctcttgcctgaaggacaggcacgacttcggcttcccacaggaggagttcggcaaccagttccagaaggccgagacaattccagtgctccacgagatgattcagcagattttcaacctgttcagcaccaaggactctagcgccgcctgggacgagacactcctcgacaagttctacaccgagctgtaccagcagctgaacgacctcgaggcctgcgtgattcagggcgtgggcgtgaccgagaccccactgatgaaggaggactctattctcgccgtgagaaagtacttccagcgcattacactgtacctcaaggagaagaagtactccccttgcgcctgggaggtggtgcgcgccgagattatgagatctttcagcctgagcaccaacctgcaggagtctctgagatctaaggagggcggcggcggctctggcggcggcggctctggcggcggcggcagcgagaagccatctccatgccagtgcagcagactgtctcctcacaaccgcacaaactgcggcttcccaggcattacatccgaccagtgcttcgacaacggctgctgcttcgactctagcgtgacaggcgtgccttggtgcttccacccactgccaaagcaggagtccgaccagtgcgtgatggaggtgagcgaccgccggaactgcggctaccccggcattagccccgaggagtgcgcctcccggaagtgctgcttcagcaacttcattttcgaggtgccttggtgcttcttccctaagtctgtggaggactgccactacgagccaaagtcttgcgacaagacccacacatgccctccatgccccgcccccgagctcctgggcggcccatctgtgttcctgttcccacctaagccaaaggacacactcatgattagccgcaccccagaggtgacatgcgtggtggtggacgtgtctcacgaggaccccgaggtgaagttcaactggtacgtggacggcgtggaggtgcacaacgccaagacaaagcctagagaggagcagtacaacagcacataccgggtggtgtccgtgctgacagtgctgcaccaggactggctgaacggcaaggagtacaagtgcaaggtgtctaacaaggccctccccgcccctattgagaagaccatttctaaggccaagggccagcctagagagcctcaggtgtacacactgccacctagccgggacgagctcacaaagaaccaggtgtccctgacatgcctcgtgaagggcttctaccctagcgacatcgccgtggagtgggagtctaacggccagccagagaacaactacaagaccaccccacccgtgctcgactccgacggctctttcttcctgtactctaagctgacagtggacaagagcagatggcagcagggcaacgtgttctcttgctctgtgatgcacgaggccctgcacaaccactacacacagaagtccctgtccctgtctcctggcaag

SEQ ID NO: 6 - protein, 518 aa, Artificial
  IFNα2-G4S-TFF2-Fc amino acid sequence
CDLPQTHSLGSRRTLMLLAQMRRISLFSCLKDRHDFGFPQEEFGNQFQKAETIPVLHEMIQQIFNLFSTKDSSAAWDETLLDKFYTELYQQLNDLEACVIQGVGVTETPLMKEDSILAVRKYFQRITLYLKEKKYSPCAWEVVRAEIMRSFSLSTNLQESLRSKEGGGGSGGGGSGGGGSEKPSPCQCSRLSPHNRTNCGFPGITSDQCFDNGCCFDSSVTGVPWCFHPLPKQESDQCVMEVSDRRNCGYPGISPEECASRKCCFSNFIFEVPWCFFPKSVEDCHYEPKSCDKTHTCPPCPAPELLGGPSVFLFPPKPKDTLMISRTPEVTCVVVDVSHEDPEVKFNWYVDGVEVHNAKTKPREEQYNSTYRVVSVLTVLHQDWLNGKEYKCKVSNKALPAPIEKTISKAKGQPREPQVYTLPPSRDELTKNQVSLTCLVKGFYPSDIAVEWESNGQPENNYKTTPPVLDSDGSFFLYSKLTVDKSRWQQGNVFSCSVMHEALHNHYTQKSLSLSPGK

SEQ ID NO: 7 - DNA, 390 bp, Homo sapiens
atgggacggcgagacgcccagctcctggcagcgctcctcgtcctggggctatgtgccctggcggggagtgagaaaccctccccctgccagtgctccaggctgagcccccataacaggacgaactgcggcttccctggaatcaccagtgaccagtgttttgacaatggatgctgtttcgactccagtgtcactggggtcccctggtgtttccaccccctcccaaagcaagagtcggatcagtgcgtcatggaggtctcagaccgaagaaactgtggctacccgggcatcagccccgaggaatgcgcctctcggaagtgctgcttctccaacttcatctttgaagtgccctggtgcttcttcccgaagtctgtggaagactgccattactaa

SEQ ID NO: 8 - protein, 129 aa, Homo sapiens
MGRRDAQLLAALLVLGLCALAGSEKPSPCQCSRLSPHNRTNCGFPGITSDQCFDNGCCFDSSVTGVPWCFHPLPKQESDQCVMEVSDRRNCGYPGISPEECASRKCCFSNFIFEVPWCFFPKSVEDCHY

SEQ ID NO: 9 - DNA, 495 bp, Homo sapiens
tgcgacctcccacagacccactctctgggctctcgcagaacactgatgctcctcgcccagatgagacggattagcctgttctcttgcctcaaggacaggcacgacttcggcttccctcaggaggagttcggcaaccagttccagaaggccgagaccattccagtgctgcacgagatgattcagcagattttcaacctgttcagcaccaaggactctagcgccgcctgggacgagaccctcctcgacaagttctacacagagctgtaccagcagctgaacgacctcgaggcctgcgtgattcagggcgtgggcgtgacagagaccccactcatgaaggaggactccattctggccgtgagaaagtacttccagcgcattacactgtacctgaaggagaagaagtactctccatgcgcctgggaggtggtgcgcgccgagattatgagatctttcagcctgagcacaaacctgcaggagtccctcagatctaaggag

SEQ ID NO: 10 - protein, 188 aa, Homo sapiens
MALTFALLVALLVLSCKSSCSVGCDLPQTHSLGSRRTLMLLAQMRRISLFSCLKDRHDFGFPQEEFGNQFQKAETIPVLHEMIQQIFNLFSTKDSSAAWDETLLDKFYTELYQQLNDLEACVIQGVGVTETPLMKEDSILAVRKYFQRITLYLKEKKYSPCAWEVVRAEIMRSFSLSTNLQESLRSKE

SEQ ID NO: 11 - DNA, 390 bp, Mus musculus
atgcgacctcgaggtgcccccctgctggcagtggtcctggttttgggactgcatgctctggtagagggcgagaaaccttccccctgtcggtgctccaggctgacaccccacaacagaaagaactgtggcttcccgggcatcaccagtgagcagtgctttgatcttggatgctgctttgactctagcgtcgctggggtcccttggtgtttccacccacttccaaaccaagaatcggagcagtgtgtcatggaagtgtcagctcgcaagaattgtgggtacccgggcatcagtcccgaggactgtgccagtcgaaactgctgcttttccaacctgatctttgaagtgccctggtgtttcttcccacagtctgtggaagattgtcactactga

SEQ ID NO: 12 - protein, 129 aa, Mus musculus
MRPRGAPLLAVVLVLGLHALVEGEKPSPCRCSRLTPHNRKNCGFPGITSEQCFDLGCCFDSSVAGVPWCFHPLPNQESEQCVMEVSARKNCGYPGISPEDCASRNCCFSNLIFEVPWCFFPQSVEDCHY

SEQ ID NO: 13 - DNA, 573 bp, Mus musculus
atggctagactctgtgctttcctcgtgatgctgatagtgatgagctactggtcaacctgttctctaggatgcgatctgcctcacacttataacctcaggaacaagagggccttgaaggtcctggcacagatgaggaggctcccctttctctcctgcctgaaggacaggcaggactttggattccccctggagaaggtggataaccagcagatccagaaggctcaagccatccctgtgctgcgagatcttactcagcagaccttgaacctcttcacatcaaaggcttcatctgctgcttggaatacaaccctcctagactcattctgcaatgacctccaccagcagctcaatgacctgcaaacctgtctgatgcagcaggtgggggtgcaggaacctcctctgacccaggaagacgccctgctggctgtgaggaaatatttccacaggatcactgtgtacctgagagagaagaaacacagcccctgtgcctgggaggtggtcagagcagaagtctggagagccctgtcttcctcagtcaacttgctgccaagactgagtgaagagaaggagtga

SEQ ID NO: 14 - protein, 190 aa, Mus musculus
MARLCAFLVMLIVMSYWSTCSLGCDLPHTYNLRNKRALKVLAQMRRLPFLSCLKDRQDFGFPLEKVDNQQIQKAQAIPVLRDLTQQTLNLFTSKASSAAWNTTLLDSFCNDLHQQLNDLQTCLMQQVGVQEPPLTQEDALLAVRKYFHRITVYLREKKHSPCAWEVVRAEVWRALSSSVNLLPRLSEEKE